European Patent Specification EP 3 101 110 B1, published August 30, 2023. Title: Enzyme and Fabric Hueing Agent Containing Compositions. Applicant: The Procter & Gamble Company. The sequence listing filed with the application follows.

SEQUENCE LISTING (2 sequences)

SEQ ID NO: 1 - DNA, 807 bp, Thermomyces lanuginosus
  CDS (1)..(807)
  mat_peptide (1)..()
gaggtctcgcaggatctgtttaaccagttcaatctctttgcacagtattctgcagccgcatactgcggaaaaaacaatgatgccccagctggtacaaacattacgtgcacgggaaatgcctgccccgaggtagagaaggcggatgcaacgtttctctactcgtttgaagactctggagtgggcgatgtcaccggcttccttgctctcgacaacacgaacaaattgatcgtcctctctttccgtggctctcgttccatagagaactggatcgggaatcttaacttcgacttgaaagaaataaatgacatttgctccggctgcaggggacatgacggcttcacttcgtcctggaggtctgtagccgatacgttaaggcagaaggtggaggatgctgtgagggagcatcccgactatcgcgtggtgtttaccggacatagcttgggtggtgcattggcaactgttgccggagcagacctgcgtggaaatgggtatgatatcgacgtgttttcatatggcgccccccgagtcggaaacagggcttttgcagaattcctgaccgtacagaccggcggaacactctaccgcattacccacaccaatgatattgtccctagactcccgccgcgcgaattcggttacagccattctagcccagagtactggatcaaatctggaacccttgtccccgtcacccgaaacgatatcgtgaagatagaaggcatcgatgccaccggcggcaataaccagcctaacattccggatatccctgcgcacctatggtacttcgggttaattgggacatgtctt

SEQ ID NO: 2 - protein, 269 aa, Thermomyces lanuginosus [sequence omitted]